European Patent Application EP 4 477 760 A1, published December 18, 2024. Title: Kit for Assaying AFP mRNA for Liver Cancer Diagnosis. Applicant: Sun Yat-Sen University Cancer Center (Affiliated Cancer Hospital of Sun Yat-Sen University, Cancer Research Institute of Sun Yat-Sen University). The sequence listing filed with the application follows.

SEQUENCE LISTING (31 sequences)

SEQ ID NO: 1 - DNA, 44 bp, synthetic construct
  source 1..44: mol_type = other DNA
tgcagtacattggtaagaatccaatatgtattatgagaaagttg

SEQ ID NO: 2 - DNA, 44 bp, synthetic construct
  source 1..44: mol_type = other DNA
tggtagccaggtcagctaaacttatctctattatgagaaagttg

SEQ ID NO: 3 - DNA, 44 bp, synthetic construct
  source 1..44: mol_type = other DNA
gcttcttgaacaaactgggcaaaaaatatattatgagaaagttg

SEQ ID NO: 4 - DNA, 44 bp, synthetic construct
  source 1..44: mol_type = other DNA
caccattttgcttacttccttgtaagtgtattatgagaaagttg

SEQ ID NO: 5 - DNA, 44 bp, synthetic construct
  source 1..44: mol_type = other DNA
gtttctcaattgcagtcaatgcatcttttattatgagaaagttg

SEQ ID NO: 6 - DNA, 44 bp, synthetic construct
  source 1..44: mol_type = other DNA
caccctgaagactgttcatctccagtggtattatgagaaagttg

SEQ ID NO: 7 - DNA, 44 bp, synthetic construct
  source 1..44: mol_type = other DNA
cagaaaggcaggtagctggttttctaaatattatgagaaagttg

SEQ ID NO: 8 - DNA, 44 bp, synthetic construct
  source 1..44: mol_type = other DNA
aaatttctttctcatggcaaagttcttctattatgagaaagttg

SEQ ID NO: 9 - DNA, 44 bp, synthetic construct
  source 1..44: mol_type = other DNA
cagcagtctgaatgtccgtacttctccatattatgagaaagttg

SEQ ID NO: 10 - DNA, 44 bp, synthetic construct
  source 1..44: mol_type = other DNA
gttatgtcttccctcttcactttggctgtattatgagaaagttg

SEQ ID NO: 11 - DNA, 44 bp, synthetic construct
  source 1..44: mol_type = other DNA
gagtgggctttttgtgtgcaagaaaacatattatgagaaagttg

SEQ ID NO: 12 - DNA, 44 bp, synthetic construct
  source 1..44: mol_type = other DNA
ggaacttggaaaagtgggatcgatgctgtattatgagaaagttg

SEQ ID NO: 13 - DNA, 44 bp, synthetic construct
  source 1..44: mol_type = other DNA
atatgcttcacagcttgtgacaggttcttattatgagaaagttg

SEQ ID NO: 14 - DNA, 44 bp, synthetic construct
  source 1..44: mol_type = other DNA
tgttcatgaatgtctccctgtcttcttctattatgagaaagttg

SEQ ID NO: 15 - DNA, 44 bp, synthetic construct
  source 1..44: mol_type = other DNA
tgccttcttgctatctcataaatgaatttattatgagaaagttg

SEQ ID NO: 16 - DNA, 44 bp, synthetic construct
  source 1..44: mol_type = other DNA
aagaattgtaggtgcatacaggaagggatattatgagaaagttg

SEQ ID NO: 17 - DNA, 44 bp, synthetic construct
  source 1..44: mol_type = other DNA
ttattttgtcatagcgagcagcccaaagtattatgagaaagttg

SEQ ID NO: 18 - DNA, 44 bp, synthetic construct
  source 1..44: mol_type = other DNA
gcattttcagctttgcagcaagatggaatattatgagaaagttg

SEQ ID NO: 19 - DNA, 44 bp, synthetic construct
  source 1..44: mol_type = other DNA
tgctgcctttgtttggaagcattcaacttattatgagaaagttg

SEQ ID NO: 20 - DNA, 44 bp, synthetic construct
  source 1..44: mol_type = other DNA
tgctttctcttaattcttttgtaactgttattatgagaaagttg

SEQ ID NO: 21 - DNA, 44 bp, synthetic construct
  source 1..44: mol_type = other DNA
actgcacatgcatgttgatttaacaagctattatgagaaagttg

SEQ ID NO: 22 - DNA, 44 bp, synthetic construct
  source 1..44: mol_type = other DNA
gaaagttcgggtcccaaaatttttcatttattatgagaaagttg

SEQ ID NO: 23 - DNA, 44 bp, synthetic construct
  source 1..44: mol_type = other DNA
gactcagtttagtaacagttatggcttgtattatgagaaagttg

SEQ ID NO: 24 - DNA, 44 bp, synthetic construct
  source 1..44: mol_type = other DNA
tcagtaaaattaactttggtaaacttcttattatgagaaagttg

SEQ ID NO: 25 - DNA, 44 bp, synthetic construct
  source 1..44: mol_type = other DNA
ggccacatccaggactagtttctggatttattatgagaaagttg

SEQ ID NO: 26 - DNA, 44 bp, synthetic construct
  source 1..44: mol_type = other DNA
ctcctctgcaacagtgctcatgtacatgtattatgagaaagttg

SEQ ID NO: 27 - DNA, 44 bp, synthetic construct
  source 1..44: mol_type = other DNA
tccccatcctgcagacaatccagcacattattatgagaaagttg

SEQ ID NO: 28 - DNA, 44 bp, synthetic construct
  source 1..44: mol_type = other DNA
ttgagaacatatgtaggacatgattttttattatgagaaagttg

SEQ ID NO: 29 - DNA, 44 bp, synthetic construct
  source 1..44: mol_type = other DNA
ctgttattttgtttgacagagtgtcttgtattatgagaaagttg

SEQ ID NO: 30 - DNA, 44 bp, synthetic construct
  source 1..44: mol_type = other DNA
cgttccagcgtggtcagtttgcagcatttattatgagaaagttg

SEQ ID NO: 31 - DNA, 16 bp, synthetic construct
  source 1..16: mol_type = other DNA
tattatgagaaagttg